European Patent Specification EP 3 777 528 B1, published November 27, 2024. Title: A non-human vertebrate animal to which human hepatocytes have been transplanted, and a method of producing the animal. Applicant: Central Institute for Experimental animals. The sequence listing filed with the application follows.

SEQUENCE LISTING (4 sequences)

SEQ ID NO: 1 - DNA, 1131 bp, Herpes simplex virus
  CDS (1)..(1131)
atggcttcgtaccccggccatcaacacgcgtctgcgttcgaccaggctgcgcgttctcgcggccatagcaaccgacgtacggcgttgcgccctcgccggcagcaagaagccacggaagtccgcccggagcagaaaatgcccacgctactgcgggtttatatagacggtccccacgggatggggaaaaccaccaccacgcaactgctggtggccctgggttcgcgcgacgatatcgtctacgtacccgagccgatgacttactggcgggtgctgggggcttccgagacaatcgcgaacatctacaccacacaacaccgcctcgaccagggtgagatatcggccggggacgcggcggtggtaatgacaagcgcccagataacaatgggcatgccttatgccgtgaccgacgccgttctggctcctcatatcgggggggaggctgggagctcacatgtcccgcccccggccctcaccattttggctgaccgccatcccatcgcatatttcttatgctacccggccgcgcggtaccttatgggcagcatgaccccccaggccgtgctggcgttcgtggccctcatcccgccgaccttgcccggcaccaacatcgtgcttggggcccttccggaggacagacacatcgaccgcctggccaaacgccagcgccccggcgagcggctggacctggctatgctggctgcgattcgccgcgtttacgggctacttgccaatacggtgcggtatctgcagtgcggcgggtcgtggcgggaggactggggacagctttcggggacggccgtgccgccccagggtgccgagccccagagcaacgcgggcccacgaccccatatcggggacacgttatttaccctgtttcgggcccccgagttgctggcccccaacggcgacctgtataacgtgtttgcctgggccttggacgtcttggccaaacgcctccgttccatgcacgtctttatcctggattacgaccaatcgcccgccggctgccgggacgccctgctgcaacttacctccgggatggtccagacccacgtcaccacccccggctccataccgacgatatgcgacctggcgcgcacgtttgcccgggagatgggggaggctaactga

SEQ ID NO: 2 - protein, 376 aa, Herpes simplex virus
MASYPGHQHASAFDQAARSRGHSNRRTALRPRRQQEATEVRPEQKMPTLLRVYIDGPHGMGKTTTTQLLVALGSRDDIVYVPEPMTYWRVLGASETIANIYTTQHRLDQGEISAGDAAVVMTSAQITMGMPYAVTDAVLAPHIGGEAGSSHVPPPALTILADRHPIAYFLCYPAARYLMGSMTPQAVLAFVALIPPTLPGTNIVLGALPEDRHIDRLAKRQRPGERLDLAMLAAIRRVYGLLANTVRYLQCGGSWREDWGQLSGTAVPPQGAEPQSNAGPRPHIGDTLFTLFRAPELLAPNGDLYNVFAWALDVLAKRLRSMHVFILDYDQSPAGCRDALLQLTSGMVQTHVTTPGSIPTICDLARTFAREMGEAN

SEQ ID NO: 3 - DNA, 1131 bp, Herpes simplex virus
  CDS (1)..(1131)
atggcttcgtacccctgccatcaacacgcgtctgcgttcgaccaggctgcgcgttctcgcggccatagcaaccgacgtacggcgttgcgccctcgccggcagcaagaagccacggaagtccgcctggagcagaaaatgcccacgctactgcgggtttatatagacggtcctcacgggatggggaaaaccaccaccacgcaactgctggtggccctgggttcgcgcgacgatatcgtctacgtacccgagccgatgacttactggcaggtgctgggggcttccgagacaatcgcgaacatctacaccacacaacaccgcctcgaccagggtgagatatcggccggggacgcggcggtggtaatgacaagcgcccagataacaatgggcatgccttatgccgtgaccgacgccgttctggctcctcatatcgggggggaggctgggagctcacatgccccgcccccggccctcaccctcatcttcgaccgccatcccatcgccgccctcctgtgctacccggccgcgcgataccttatgggcagcatgaccccccaggccgtgctggcgttcgtggccctcatcccgccgaccttgcccggcacaaacatcgtgttgggggcccttccggaggacagacacatcgaccgcctggccaaacgccagcgccccggcgagcggcttgacctggctatgctggccgcgattcgccgcgtttacgggctgcttgccaatacggtgcggtatctgcagggcggcgggtcgtggcgggaggattggggacagctttcggggacggccgtgccgccccagggtgccgagccccagagcaacgcgggcccacgaccccatatcggggacacgttatttaccctgtttcgggcccccgagttgctggcccccaacggcgacctgtacaacgtgtttgcctgggccttggacgtcttggccaaacgcctccgtcccatgcacgtctttatcctggattacgaccaatcgcccgccggctgccgggacgccctgctgcaacttacctccgggatggtccagacccacgtcaccacccccggctccataccgacgatctgcgacctggcgcgcacgtttgcccgggagatgggggaggctaactga

SEQ ID NO: 4 - protein, 376 aa, Herpes simplex virus
MASYPCHQHASAFDQAARSRGHSNRRTALRPRRQQEATEVRLEQKMPTLLRVYIDGPHGMGKTTTTQLLVALGSRDDIVYVPEPMTYWQVLGASETIANIYTTQHRLDQGEISAGDAAVVMTSAQITMGMPYAVTDAVLAPHIGGEAGSSHAPPPALTLIFDRHPIAALLCYPAARYLMGSMTPQAVLAFVALIPPTLPGTNIVLGALPEDRHIDRLAKRQRPGERLDLAMLAAIRRVYGLLANTVRYLQGGGSWREDWGQLSGTAVPPQGAEPQSNAGPRPHIGDTLFTLFRAPELLAPNGDLYNVFAWALDVLAKRLRPMHVFILDYDQSPAGCRDALLQLTSGMVQTHVTTPGSIPTICDLARTFAREMGEAN